European Patent Specification EP 3 820 899 B1, published March 5, 2025. Title: Antibody molecules. Applicant: F-star Beta Limited. Application WO. The sequence listing filed with the application follows.

SEQUENCE LISTING (184 sequences)

SEQ ID NO: 1 - protein, 5 aa, Artificial Sequence
  HCDR1 (Kabat)
SYGIS

SEQ ID NO: 2 - protein, 17 aa, Artificial Sequence
  HCDR2 formula (Kabat)
  MISC_FEATURE (6)..(6): Xaa is Ser, Asn, or Gly
  MISC_FEATURE (7)..(7): Xaa is is Gly or Ser
  MISC_FEATURE (8)..(8): Xaa is or Gly, Asn or Ser
  MISC_FEATURE (9)..(9): Xaa is Thr or Ala
WISAYXXXXNYAQKLQG

SEQ ID NO: 3 - protein, 14 aa, Artificial Sequence
  HCDR3 (Kabat)
DLFPTIFGVSYYYY

SEQ ID NO: 4 - protein, 4 aa, Artificial Sequence
  Formula for residues 54-57 (X1 to X4)(Kabat) and residues 62-65 (X2 to X5) (IMGT) of HCDR2
  MISC_FEATURE (1)..(1): Xaa selected from Ser, Asn and Gly
  MISC_FEATURE (2)..(2): Xaa selected from Gly and Ser
  MISC_FEATURE (3)..(3): Xaa selected from Gly, Asn and Ser
  MISC_FEATURE (4)..(4): Xaa selected from Thr and Ala
XXXX

SEQ ID NO: 5 - protein, 4 aa, Artificial Sequence
  Residues 54-57 of HCDR2 (Kabat) of G1/929_01_A02, G1/929_01_A05, G1/929_01_A08, G1/929_01_A11.
SGGT

SEQ ID NO: 6 - protein, 4 aa, Artificial Sequence
  Residues 54-57 of HCDR2 (Kabat) of G1/887_04_E12 (Parent), G1/894_08_A05 (Parent), G1/894_08_E05 (Parent) and G1/887_04_G12 (Parent).
NSNT

SEQ ID NO: 7 - protein, 4 aa, Artificial Sequence
  Residues 54-57 of HCDR2 (Kabat) of G1/929_01_A01, G1/929_01_A04, G1/929_01_A07 and G1/929_01_A10.
GGST

SEQ ID NO: 8 - protein, 4 aa, Artificial Sequence
  Residues 54-57 of HCDR2 (Kabat) of G1/929_01_A03, G1/929_01_A06, G1/929_01_A09 and G1/929_01_A12.
SGNA

SEQ ID NO: 9 - protein, 11 aa, Artificial Sequence
  Formula for kappa VL LCDR1 (Kabat)
  MISC_FEATURE (7)..(7): Xaa is Gly or Ser
  MISC_FEATURE (8)..(8): Xaa is Asn or Gly
RASQSIXXRLA

SEQ ID NO: 10 - protein, 7 aa, Artificial Sequence
  Formula for kappa VL LCDR2 (Kabat)
  MISC_FEATURE (4)..(4): Xaa is Thr or Asn
  MISC_FEATURE (5)..(5): Xaa is Ser or Leu
  MISC_FEATURE (7)..(7): Xaa is Thr or Ser
EASXXEX

SEQ ID NO: 11 - protein, 10 aa, Artificial Sequence
  Formula for kappa VL LCDR3 (Kabat)
  MISC_FEATURE (3)..(3): Xaa is Ser or Ala
  MISC_FEATURE (4)..(4): Xaa is Tyr or Asn
  MISC_FEATURE (5)..(5): Xaa is Ser or Thr
  MISC_FEATURE (6)..(6): Xaa is Thr, Trp or Phe
  MISC_FEATURE (8)..(8): Xaa is absent or Arg
  MISC_FEATURE (9)..(9): Xaa is Tyr, Arg or Val
  MISC_FEATURE (10)..(10): Xaa is Thr or Ser
QQXXXXPXXX

SEQ ID NO: 12 - protein, 14 aa, Artificial Sequence
  Formula for Lambda VL LCDR1 (Kabat)
  MISC_FEATURE (12)..(12): Xaa is Tyr or Ser
TGTSSDVGGYNXVS

SEQ ID NO: 13 - protein, 7 aa, Artificial Sequence
  Lambda VL LCDR2 (Kabat) G1/280_02_G02, G1/280_02_G02_NS, G1AA/lambdav3.
EVTNRPS

SEQ ID NO: 14 - protein, 11 aa, Artificial Sequence
  Lambda VL LCDR3 (Kabat and IMGT) of G1/280_02_G02, G1/280_02_G02_NS and G1AA/lambdav3
SSFKRGSTLVV

SEQ ID NO: 15 - protein, 11 aa, Artificial Sequence
  Kappa VL LCDR1 (Kabat) G1/887_04_E12, G1AA/E12v2, G1/929_01_A01, G1/929_01_A02, G1/929_01_A03.
RASQSIGNRLA

SEQ ID NO: 16 - protein, 7 aa, Artificial Sequence
  Kappa VL LCDR2 (Kabat) of G1/887_04_E12, G1AA/E12v2, G1/929_01_A02, G1/929_01_A03,
EASTSET

SEQ ID NO: 17 - protein, 9 aa, Artificial Sequence
  Kappa VL LCDR3 (Kabat and IMGT) of G1/887_04_E12, G1AA/E12v2, G1/929_01_A01, G1/929_01_A02 and G1/929_01_A03.
QQSYSTPYT

SEQ ID NO: 18 - protein, 17 aa, Artificial Sequence
  VH HCDR2 (Kabat) of G1AA/E05v2, G1AA/E12v2, G1AA/G12v2, G1AA/lambdav3,  G1/929_01_A08, G1/929_01_A02, G1/929_01_A11 and G1/929_01_A05.
WISAYSGGTNYAQKLQG

SEQ ID NO: 19 - protein, 11 aa, Artificial Sequence
  VL LCDR1 (Kabat) G1/894_08_E05, G1/887_04_G12, G1/894_08_A05, G1AA/E05v2, G1AA/G12v2, G1/929_01_A07, G1/929_01_A08, G1/929_01_A09, G1/929_01_A10, G1/929_01_A11, G1/929_01_A12, G1/929_01_A04, G1/929_01_A05, G1/929_01_A06.
RASQSISGRLA

SEQ ID NO: 20 - protein, 7 aa, Artificial Sequence
  VL LCDR2 (Kabat) G1/894_08_E05, G1/887_04_G12, G1/894_08_A05, G1AA/E05v2, G1AA/G12v2, G1/929_01_A07, G1/929_01_A08, G1/929_01_A09, G1/929_01_A10, G1/929_01_A11, G1/929_01_A12, G1/929_01_A04, G1/929_01_A05, G1/929_01_A06
EASNLES

SEQ ID NO: 21 - protein, 9 aa, Artificial Sequence
  VL LCDR3 (Kabat and IMGT) G1/887_04_G12, G1AA/G12v2, G1/929_01_A10, G1/929_01_A11, G1/929_01_A12.
QQSYSWPRT

SEQ ID NO: 22 - protein, 10 aa, Artificial Sequence
  VL LCDR3 (Kabat and IMGT) G1/894_08_E05, G1AA/E05v2, G1/929_01_A07, G1/929_01_A08, G1/929_01_A09.
QQSYSTPRVT

SEQ ID NO: 23 - protein, 17 aa, Artificial Sequence
  VH HCDR2 (Kabat) G1/280_02_G02_NS, G1/894_08_E05, G1/887_04_E12, G1/887_04_G12, G1/894_08_A05.
WISAYNSNTNYAQKLQG

SEQ ID NO: 24 - protein, 10 aa, Artificial Sequence
  VL LCDR3 (Kabat and IMGT) of G1/894_08_A05,  G1/929_01_A04, G1/929_01_A05, G1/929_01_A06
QQANTFPRVS

SEQ ID NO: 25 - protein, 14 aa, Artificial Sequence
  VL LCDR1 (Kabat) G1AA/lambdav3
TGTSSDVGGYNYVS

SEQ ID NO: 26 - protein, 14 aa, Artificial Sequence
  VL LCDR1 (Kabat) of G1/280_02_G02 and G1/280_02_G02_NS
TGTSSDVGGYNSVS

SEQ ID NO: 27 - protein, 123 aa, Artificial Sequence
  VH domain of G1AA/E12v2
EVQLVQSGAEVKRPGASVKVSCKASGYPFTSYGISWVRQAPGQGLEWMGWISAYSGGTNYAQKLQGRVTMTTDTSTSTAYMELRSLRSDDTAVYYCARDLFPTIFGVSYYYYWGQGTLVTVSS

SEQ ID NO: 28 - protein, 107 aa, Artificial Sequence
  VL domain of G1AA/E12v2
DIQMTQSPSTLSASVRDRVIITCRASQSIGNRLAWYQHKPGKAPKLLIYEASTSETGVPSRFSGSGSGTDFTLTISSLQPEDFATYYCQQSYSTPYTFGQGTKLEIK

SEQ ID NO: 29 - protein, 123 aa, Artificial Sequence
  VH domain of G1AA/G12v2
EVQLVQSGAEVKRPGASVKVSCKASGYTFTSYGISWVRQAPGQGLEWMGWISAYSGGTNYAQKLQGRVTMTTDTSTSTAYMELRSLRSDDTAVYYCARDLFPTIFGVSYYYYWGQGTLVTVSS

SEQ ID NO: 30 - protein, 107 aa, Artificial Sequence
  VL domain of G1AA/G12v2
DIQMTQSPSTLSASVGDRVTITCRASQSISGRLAWYQQKPGKAPNLLIYEASNLESGVPSRFSGSGSGTEFTLTISSLQPEDFATYYCQQSYSWPRTFGQGTKVEIK

SEQ ID NO: 31 - protein, 123 aa, Artificial Sequence; identical to SEQ ID NO: 29
  VH domain of G1AA/E05v2

SEQ ID NO: 32 - protein, 108 aa, Artificial Sequence
  VL domain of G1AA/E05v2
DIQMTQSPSTLSASVGDRVTITCRASQSISGRLAWYQQKPGKAPNLLIYEASNLESGVPSRFSGSGSGTEFTLTISSLQPEDFATYYCQQSYSTPRVTFGQGTKVEIK

SEQ ID NO: 33 - protein, 123 aa, Artificial Sequence
  VH domain of G1/887_04_E12
EVQLVQSGAEVKRPGASVKVSCKASGYPFTSYGISWVRQAPGQGLEWMGWISAYNSNTNYAQKLQGRVTMTTDTSTSTAYMELRSLRSDDTAVYYCARDLFPTIFGVSYYYYWGQGTLVTVSS

SEQ ID NO: 34 - protein, 107 aa, Artificial Sequence; identical to SEQ ID NO: 28
  VL of antibody G1/887_04_E12

SEQ ID NO: 35 - protein, 123 aa, Artificial Sequence
  VH domain of G1/887_04_G12
EVQLVQSGAEVKRPGASVKVSCKASGYTFTSYGISWVRQAPGQGLEWMGWISAYNSNTNYAQKLQGRVTMTTDTSTSTAYMELRSLRSDDTAVYYCARDLFPTIFGVSYYYYWGQGTLVTVSS

SEQ ID NO: 36 - protein, 107 aa, Artificial Sequence; identical to SEQ ID NO: 30
  VL domain of G1/887_04_G12

SEQ ID NO: 37 - protein, 123 aa, Artificial Sequence; identical to SEQ ID NO: 35
  VH domain of G1/894_08_E05

SEQ ID NO: 38 - protein, 108 aa, Artificial Sequence; identical to SEQ ID NO: 32
  VL domain of G1/894_08_E05

SEQ ID NO: 39 - protein, 123 aa, Artificial Sequence; identical to SEQ ID NO: 35
  VH domain of G1/894_08_A05

SEQ ID NO: 40 - protein, 108 aa, Artificial Sequence
  VL domain of G1/894_08_A05
DIQMTQSPSTLSASVGDRVTITCRASQSISGRLAWYQQKPGKAPNLLIYEASNLESGVPSRFSGSGSGTEFTLTINSLQPDDFATYYCQQANTFPRVSFGGGTKVEIK

SEQ ID NO: 41 - protein, 123 aa, Artificial Sequence; identical to SEQ ID NO: 29
  VH domain of G1AA/lambdav3

SEQ ID NO: 42 - protein, 111 aa, Artificial Sequence
  VL domain of G1AA/lambdav3
QSALTQPASVSGSPGQSITISCTGTSSDVGGYNYVSWYQQFPGKAPKLMIFEVTNRPSGVSDRFSGSKSDNTASLTISGLQAEDEAEYYCSSFKRGSTLVVFGGGTKLTVL

SEQ ID NO: 43 - protein, 123 aa, Artificial Sequence; identical to SEQ ID NO: 35
  VH domain of G1/280_02_G02_NS

SEQ ID NO: 44 - protein, 111 aa, Artificial Sequence
  VL domain of G1/280_02_G02_NS
QSALTQPASVSGSPGQSITISCTGTSSDVGGYNSVSWYQQFPGKAPKLMIFEVTNRPSGVSDRFSGSKSDNTASLTISGLQAEDEAEYYCSSFKRGSTLVVFGGGTKLTVL

SEQ ID NO: 45 - protein, 123 aa, Artificial Sequence
  VH domain of G1/280_02_G02
EVQLVQSGAEVKRPGASVKVSCKASGYTFTSYGISWVRQAPGQGLEWMGWISAYNGNTNYAQKLQGRVTMTTDTSTSTAYMELRSLRSDDTAVYYCARDLFPTIFGVSYYYYWGQGTLVTVSS

SEQ ID NO: 46 - protein, 111 aa, Artificial Sequence; identical to SEQ ID NO: 44
  VL domain of G1/280_02_G02

SEQ ID NO: 47 - protein, 452 aa, Artificial Sequence
  G1AA/E12v2  IgG1 heavy chain with LALA
EVQLVQSGAEVKRPGASVKVSCKASGYPFTSYGISWVRQAPGQGLEWMGWISAYSGGTNYAQKLQGRVTMTTDTSTSTAYMELRSLRSDDTAVYYCARDLFPTIFGVSYYYYWGQGTLVTVSSASTKGPSVFPLAPSSKSTSGGTAALGCLVKDYFPEPVTVSWNSGALTSGVHTFPAVLQSSGLYSLSSVVTVPSSSLGTQTYICNVNHKPSNTKVDKKVEPKSCDKTHTCPPCPAPEAAGGPSVFLFPPKPKDTLMISRTPEVTCVVVDVSHEDPEVKFNWYVDGVEVHNAKTKPREEQYNSTYRVVSVLTVLHQDWLNGKEYKCKVSNKALPAPIEKTISKAKGQPREPQVYTLPPSRDELTKNQVSLTCLVKGFYPSDIAVEWESNGQPENNYKTTPPVLDSDGSFFLYSKLTVDKSRWQQGNVFSCSVMHEALHNHYTQKSLSLSPG

SEQ ID NO: 48 - protein, 214 aa, Artificial Sequence
  G1AA/E12v2 IgG1 light chain
DIQMTQSPSTLSASVRDRVIITCRASQSIGNRLAWYQHKPGKAPKLLIYEASTSETGVPSRFSGSGSGTDFTLTISSLQPEDFATYYCQQSYSTPYTFGQGTKLEIKRTVAAPSVFIFPPSDEQLKSGTASVVCLLNNFYPREAKVQWKVDNALQSGNSQESVTEQDSKDSTYSLSSTLTLSKADYEKHKVYACEVTHQGLSSPVTKSFNRGEC

SEQ ID NO: 49 - protein, 452 aa, Artificial Sequence
  G1AA/G12v2 IgG1 heavy chain with LALA
EVQLVQSGAEVKRPGASVKVSCKASGYTFTSYGISWVRQAPGQGLEWMGWISAYSGGTNYAQKLQGRVTMTTDTSTSTAYMELRSLRSDDTAVYYCARDLFPTIFGVSYYYYWGQGTLVTVSSASTKGPSVFPLAPSSKSTSGGTAALGCLVKDYFPEPVTVSWNSGALTSGVHTFPAVLQSSGLYSLSSVVTVPSSSLGTQTYICNVNHKPSNTKVDKKVEPKSCDKTHTCPPCPAPEAAGGPSVFLFPPKPKDTLMISRTPEVTCVVVDVSHEDPEVKFNWYVDGVEVHNAKTKPREEQYNSTYRVVSVLTVLHQDWLNGKEYKCKVSNKALPAPIEKTISKAKGQPREPQVYTLPPSRDELTKNQVSLTCLVKGFYPSDIAVEWESNGQPENNYKTTPPVLDSDGSFFLYSKLTVDKSRWQQGNVFSCSVMHEALHNHYTQKSLSLSPG

SEQ ID NO: 50 - protein, 214 aa, Artificial Sequence
  G1AA/G12v2 IgG1 light chain
DIQMTQSPSTLSASVGDRVTITCRASQSISGRLAWYQQKPGKAPNLLIYEASNLESGVPSRFSGSGSGTEFTLTISSLQPEDFATYYCQQSYSWPRTFGQGTKVEIKRTVAAPSVFIFPPSDEQLKSGTASVVCLLNNFYPREAKVQWKVDNALQSGNSQESVTEQDSKDSTYSLSSTLTLSKADYEKHKVYACEVTHQGLSSPVTKSFNRGEC

SEQ ID NO: 51 - protein, 452 aa, Artificial Sequence; identical to SEQ ID NO: 49
  G1AA/E05v2 IgG1 heavy chain with LALA

SEQ ID NO: 52 - protein, 215 aa, Artificial Sequence
  G1AA/E05v2 IgG1 light chain
DIQMTQSPSTLSASVGDRVTITCRASQSISGRLAWYQQKPGKAPNLLIYEASNLESGVPSRFSGSGSGTEFTLTISSLQPEDFATYYCQQSYSTPRVTFGQGTKVEIKRTVAAPSVFIFPPSDEQLKSGTASVVCLLNNFYPREAKVQWKVDNALQSGNSQESVTEQDSKDSTYSLSSTLTLSKADYEKHKVYACEVTHQGLSSPVTKSFNRGEC

SEQ ID NO: 53 - protein, 452 aa, Artificial Sequence
  G1/887_04_E12 IgG1 heavy chain
EVQLVQSGAEVKRPGASVKVSCKASGYPFTSYGISWVRQAPGQGLEWMGWISAYNSNTNYAQKLQGRVTMTTDTSTSTAYMELRSLRSDDTAVYYCARDLFPTIFGVSYYYYWGQGTLVTVSSASTKGPSVFPLAPSSKSTSGGTAALGCLVKDYFPEPVTVSWNSGALTSGVHTFPAVLQSSGLYSLSSVVTVPSSSLGTQTYICNVNHKPSNTKVDKKVEPKSCDKTHTCPPCPAPELLGGPSVFLFPPKPKDTLMISRTPEVTCVVVDVSHEDPEVKFNWYVDGVEVHNAKTKPREEQYNSTYRVVSVLTVLHQDWLNGKEYKCKVSNKALPAPIEKTISKAKGQPREPQVYTLPPSRDELTKNQVSLTCLVKGFYPSDIAVEWESNGQPENNYKTTPPVLDSDGSFFLYSKLTVDKSRWQQGNVFSCSVMHEALHNHYTQKSLSLSPG

SEQ ID NO: 54 - protein, 215 aa, Artificial Sequence
  G1/887_04_E12 light chain
DIQMTQSPSTLSASVRDRVIITCRASQSIGNRLAWYQHKPGKAPKLLIYEASTSETGVPSRFSGSGSGTDFTLTISSLQPEDFATYYCQQSYSTPYTFGQGTKLEIKRTAAAAPSVFIFPPSDEQLKSGTASVVCLLNNFYPREAKVQWKVDNALQSGNSQESVTEQDSKDSTYSLSSTLTLSKADYEKHKLYACEVTHQGLSSPVTKSFNRGEC

SEQ ID NO: 55 - protein, 452 aa, Artificial Sequence
  G1/887_04_G12 IgG1 heavy chain
EVQLVQSGAEVKRPGASVKVSCKASGYTFTSYGISWVRQAPGQGLEWMGWISAYNSNTNYAQKLQGRVTMTTDTSTSTAYMELRSLRSDDTAVYYCARDLFPTIFGVSYYYYWGQGTLVTVSSASTKGPSVFPLAPSSKSTSGGTAALGCLVKDYFPEPVTVSWNSGALTSGVHTFPAVLQSSGLYSLSSVVTVPSSSLGTQTYICNVNHKPSNTKVDKKVEPKSCDKTHTCPPCPAPELLGGPSVFLFPPKPKDTLMISRTPEVTCVVVDVSHEDPEVKFNWYVDGVEVHNAKTKPREEQYNSTYRVVSVLTVLHQDWLNGKEYKCKVSNKALPAPIEKTISKAKGQPREPQVYTLPPSRDELTKNQVSLTCLVKGFYPSDIAVEWESNGQPENNYKTTPPVLDSDGSFFLYSKLTVDKSRWQQGNVFSCSVMHEALHNHYTQKSLSLSPG

SEQ ID NO: 56 - protein, 215 aa, Artificial Sequence
  G1/887_04_G12 IgG1 light chain
DIQMTQSPSTLSASVGDRVTITCRASQSISGRLAWYQQKPGKAPNLLIYEASNLESGVPSRFSGSGSGTEFTLTISSLQPEDFATYYCQQSYSWPRTFGQGTKVEIKRTAAAAPSVFIFPPSDEQLKSGTASVVCLLNNFYPREAKVQWKVDNALQSGNSQESVTEQDSKDSTYSLSSTLTLSKADYEKHKLYACEVTHQGLSSPVTKSFNRGEC

SEQ ID NO: 57 - protein, 452 aa, Artificial Sequence; identical to SEQ ID NO: 55
  G1/894_08_E05 IgG1 heavy chain

SEQ ID NO: 58 - protein, 216 aa, Artificial Sequence
  G1/894_08_E05 IgG1 light chain
DIQMTQSPSTLSASVGDRVTITCRASQSISGRLAWYQQKPGKAPNLLIYEASNLESGVPSRFSGSGSGTEFTLTISSLQPEDFATYYCQQSYSTPRVTFGQGTKVEIKRTAAAAPSVFIFPPSDEQLKSGTASVVCLLNNFYPREAKVQWKVDNALQSGNSQESVTEQDSKDSTYSLSSTLTLSKADYEKHKLYACEVTHQGLSSPVTKSFNRGEC

SEQ ID NO: 59 - protein, 452 aa, Artificial Sequence; identical to SEQ ID NO: 55
  G1/894_08_A05 IgG1 heavy chain

SEQ ID NO: 60 - protein, 216 aa, Artificial Sequence
  G1/894_08_A05 IgG1 light chain
DIQMTQSPSTLSASVGDRVTITCRASQSISGRLAWYQQKPGKAPNLLIYEASNLESGVPSRFSGSGSGTEFTLTINSLQPDDFATYYCQQANTFPRVSFGGGTKVEIKRTAAAAPSVFIFPPSDEQLKSGTASVVCLLNNFYPREAKVQWKVDNALQSGNSQESVTEQDSKDSTYSLSSTLTLSKADYEKHKLYACEVTHQGLSSPVTKSFNRGEC

SEQ ID NO: 61 - protein, 452 aa, Artificial Sequence; identical to SEQ ID NO: 49
  G1AA/lambdav3 IgG1 heavy chain with LALA

SEQ ID NO: 62 - protein, 217 aa, Artificial Sequence
  G1AA/lambdav3 IgG1 light chain
QSALTQPASVSGSPGQSITISCTGTSSDVGGYNYVSWYQQFPGKAPKLMIFEVTNRPSGVSDRFSGSKSDNTASLTISGLQAEDEAEYYCSSFKRGSTLVVFGGGTKLTVLGQPAAAPSVTLFPPSSEELQANKATLVCLISDFYPGAVTVAWKADSSPVKAGVETTTPSKQSNNKYAASSYLSLTPEQWKSHRSYSCQVTHEGSTVEKTVAPTECS

SEQ ID NO: 63 - protein, 452 aa, Artificial Sequence; identical to SEQ ID NO: 55
  G1/280_02_G02_NS IgG1 heavy chain

SEQ ID NO: 64 - protein, 217 aa, Artificial Sequence
  G1/280_02_G02_NS IgG1 light chain
QSALTQPASVSGSPGQSITISCTGTSSDVGGYNSVSWYQQFPGKAPKLMIFEVTNRPSGVSDRFSGSKSDNTASLTISGLQAEDEAEYYCSSFKRGSTLVVFGGGTKLTVLGQPAAAPSVTLFPPSSEELQANKATLVCLISDFYPGAVTVAWKADSSPVKAGVETTTPSKQSNNKYAASSYLSLTPEQWKSHRSYSCQVTHEGSTVEKTVAPTECS

SEQ ID NO: 65 - protein, 452 aa, Artificial Sequence
  G1/280_02_G02 IgG1 heavy chain
EVQLVQSGAEVKRPGASVKVSCKASGYTFTSYGISWVRQAPGQGLEWMGWISAYNGNTNYAQKLQGRVTMTTDTSTSTAYMELRSLRSDDTAVYYCARDLFPTIFGVSYYYYWGQGTLVTVSSASTKGPSVFPLAPSSKSTSGGTAALGCLVKDYFPEPVTVSWNSGALTSGVHTFPAVLQSSGLYSLSSVVTVPSSSLGTQTYICNVNHKPSNTKVDKKVEPKSCDKTHTCPPCPAPELLGGPSVFLFPPKPKDTLMISRTPEVTCVVVDVSHEDPEVKFNWYVDGVEVHNAKTKPREEQYNSTYRVVSVLTVLHQDWLNGKEYKCKVSNKALPAPIEKTISKAKGQPREPQVYTLPPSRDELTKNQVSLTCLVKGFYPSDIAVEWESNGQPENNYKTTPPVLDSDGSFFLYSKLTVDKSRWQQGNVFSCSVMHEALHNHYTQKSLSLSPG

SEQ ID NO: 66 - protein, 217 aa, Artificial Sequence; identical to SEQ ID NO: 64
  G1/280_02_G02 IgG1 light chain

SEQ ID NO: 67 - protein, 8 aa, Artificial Sequence
  Formula for HCDR1 (IMGT)
  MISC_FEATURE (3)..(3): Xaa is Pro or Thr
GYXFTSYG

SEQ ID NO: 68 - protein, 8 aa, Artificial Sequence
  Formula for HCDR2 (IMGT)
  MISC_FEATURE (5)..(5): Xaa is Ser, Asn or Gly
  MISC_FEATURE (6)..(6): Xaa is Gly or Ser
  MISC_FEATURE (7)..(7): Xaa is Gly, Asn or Ser
  MISC_FEATURE (8)..(8): Xaa is Thr or Ala
ISAYXXXX

SEQ ID NO: 69 - protein, 16 aa, Artificial Sequence
  HCDR3 (IMGT) common to all clones
ARDLFPTIFGVSYYYY

SEQ ID NO: 70 - protein, 6 aa, Artificial Sequence
  Kappa VL LCDR1 formula (IMGT) QSIX6X7R
  MISC_FEATURE (4)..(4): Xaa is Gly or Ser
  MISC_FEATURE (5)..(5): Xaa is Asn or Gly
QSIXXR

SEQ ID NO: 71 - protein, 3 aa, Artificial Sequence
  Kappa VL LCDR2 (IMGT)
EAS

SEQ ID NO: 72 - protein, 9 aa, Artificial Sequence
  Formula for Kappa VL LCDR3 (QQX8X9X10TPYT) (IMGT)
  MISC_FEATURE (3)..(3): Xaa is Ser or Ala
  MISC_FEATURE (4)..(4): Xaa is Tyr or Asn
  MISC_FEATURE (5)..(5): Xaa is Ser or Thr
QQXXXTPYT

SEQ ID NO: 73 - protein, 10 aa, Artificial Sequence
  Formula for Kappa VL LCDR3 (QQX8X9X10TPRVT) (IMGT)
  MISC_FEATURE (3)..(3): Xaa is Ser or Ala
  MISC_FEATURE (4)..(4): Xaa is Tyr or Asn
  MISC_FEATURE (5)..(5): Xaa is Ser or Thr
QQXXXTPRVT

SEQ ID NO: 74 - protein, 10 aa, Artificial Sequence
  Formula for Kappa VL LCDR3 (QQX8X9X10FPRVS) (IMGT)
  MISC_FEATURE (3)..(3): Xaa is Ser or Ala
  MISC_FEATURE (4)..(4): Xaa is Tyr or Asn
  MISC_FEATURE (5)..(5): Xaa is Ser or Thr
QQXXXFPRVS

SEQ ID NO: 75 - protein, 9 aa, Artificial Sequence
  Formula for Kappa VL LCDR3 (QQX8X9X10WPRT) (IMGT)
  MISC_FEATURE (3)..(3): Xaa is Ser or Ala
  MISC_FEATURE (4)..(4): Xaa is Tyr or Asn
  MISC_FEATURE (5)..(5): Xaa is Ser or Thr
QQXXXWPRT

SEQ ID NO: 76 - protein, 9 aa, Artificial Sequence
  Formula for lambda VL LCDR1 (SSDVGGYNX11) (IMGT)
  MISC_FEATURE (9)..(9): Xaa is Tyr or Ser
SSDVGGYNX

SEQ ID NO: 77 - protein, 3 aa, Artificial Sequence
  Lambda VL LCDR2
EVT

SEQ ID NO: 78 - protein, 17 aa, Artificial Sequence
  G1/280_02_G02 HCDR2 (Kabat)
WISAYNGNTNYAQKLQG

SEQ ID NO: 79 - protein, 433 aa, Artificial Sequence
  human PD-L1-rCd4-His
MRIFAVFIFMTYWHLLNAFTVTVPKDLYVVEYGSNMTIECKFPVEKQLDLAALIVYWEMEDKNIIQFVHGEEDLKVQHSSYRQRARLLKDQLSLGNAALQITDVKLQDAGVYRCMISYGGADYKRITVKVNAPYNKINQRILVVDPVTSEHELTCQAEGYPKAEVIWTSSDHQVLSGKTTTTNSKREEKLFNVTSTLRINTTTNEIFYCTFRRLDPEENHTAELVIPELPLAHPPNERTAAATSITAYKSEGESAEFSFPLNLGEESLQGELRWKAEKAPSSQSWITFSLKNQKVSVQKSTSNPKFQLSETLPLTLQIPQVSLQFAGSGNLTLTLDRGILYQEVNLVVMKVTQPDSNTLTCEVMGPTSPKMRLILKQENQEARVSRQEKVIQVQAPEAGVWQCLLSEGEEVKMDSKIQVLSKGLNGSHHHHHH

SEQ ID NO: 80 - protein, 477 aa, Artificial Sequence
  Human PD-L1-Fc-His
MRIFAVFIFMTYWHLLNAFTVTVPKDLYVVEYGSNMTIECKFPVEKQLDLAALIVYWEMEDKNIIQFVHGEEDLKVQHSSYRQRARLLKDQLSLGNAALQITDVKLQDAGVYRCMISYGGADYKRITVKVNAPYNKINQRILVVDPVTSEHELTCQAEGYPKAEVIWTSSDHQVLSGKTTTTNSKREEKLFNVTSTLRINTTTNEIFYCTFRRLDPEENHTAELVIPELPLAHPPNERTAAADKTHTCPPCPAPELLGGPSVFLFPPKPKDTLMISRTPEVTCVVVDVSHEDPEVKFNWYVDGVEVHNAKTKPREEQYNSTYRVVSVLTVLHQDWLNGKEYKCKVSNKALPAPIEKTISKAKGQPREPQVYTLPPSRDELTKNQVSLTCLVKGFYPSDIAVEWESNGQPENNYKTTPPVLDSDGSFFLYSKLTVDKSRWQQGNVFSCSVMHEALHNHYTQKSLSLSPGKGSHHHHHH

SEQ ID NO: 81 - protein, 432 aa, Artificial Sequence
  Mouse PD-L1-rCD4-His
MRIFAGIIFTACCHLLRAFTITAPKDLYVVEYGSNVTMECRFPVERELDLLALVVYWEKEDEQVIQFVAGEEDLKPQHSNFRGRASLPKDQLLKGNAALQITDVKLQDAGVYCCIISYGGADYKRITLKVNAPYRKINQRISVDPATSEHELICQAEGYPEAEVIWTNSDHQPVSGKRSVTTSRTEGMLLNVTSSLRVNATANDVFYCTFWRSQPGQNHTAELIIPELPATHPPQNRTAAATSITAYKSEGESAEFSFPLNLGEESLQGELRWKAEKAPSSQSWITFSLKNQKVSVQKSTSNPKFQLSETLPLTLQIPQVSLQFAGSGNLTLTLDRGILYQEVNLVVMKVTQPDSNTLTCEVMGPTSPKMRLILKQENQEARVSRQEKVIQVQAPEAGVWQCLLSEGEEVKMDSKIQVLSKGLNGSHHHHHH

SEQ ID NO: 82 - protein, 476 aa, Artificial Sequence
  Mouse PD-L1-Fc-His
MRIFAGIIFTACCHLLRAFTITAPKDLYVVEYGSNVTMECRFPVERELDLLALVVYWEKEDEQVIQFVAGEEDLKPQHSNFRGRASLPKDQLLKGNAALQITDVKLQDAGVYCCIISYGGADYKRITLKVNAPYRKINQRISVDPATSEHELICQAEGYPEAEVIWTNSDHQPVSGKRSVTTSRTEGMLLNVTSSLRVNATANDVFYCTFWRSQPGQNHTAELIIPELPATHPPQNRTAAADKTHTCPPCPAPELLGGPSVFLFPPKPKDTLMISRTPEVTCVVVDVSHEDPEVKFNWYVDGVEVHNAKTKPREEQYNSTYRVVSVLTVLHQDWLNGKEYKCKVSNKALPAPIEKTISKAKGQPREPQVYTLPPSRDELTKNQVSLTCLVKGFYPSDIAVEWESNGQPENNYKTTPPVLDSDGSFFLYSKLTVDKSRWQQGNVFSCSVMHEALHNHYTQKSLSLSPGKGSHHHHHH

SEQ ID NO: 83 - protein, 272 aa, Homo sapiens
FTVTVPKDLYVVEYGSNMTIECKFPVEKQLDLAALIVYWEMEDKNIIQFVHGEEDLKVQHSSYRQRARLLKDQLSLGNAALQITDVKLQDAGVYRCMISYGGADYKRITVKVNAPYNKINQRILVVDPVTSEHELTCQAEGYPKAEVIWTSSDHQVLSGKTTTTNSKREEKLFNVTSTLRINTTTNEIFYCTFRRLDPEENHTAELVIPELPLAHPPNERTHLVILGAILLCLGVALTFIFRLRKGRMMDVKKCGIQDTNSKKQSDTHLEET

SEQ ID NO: 84 - protein, 272 aa, Mus musculus [sequence omitted]

SEQ ID NO: 85 - protein, 457 aa, Artificial Sequence
  FS22-172-003AA/G12v2 mAb2 heavy chain with LALA
EVQLVQSGAEVKRPGASVKVSCKASGYPFTSYGISWVRQAPGQGLEWMGWISAYSGGTNYAQKLQGRVTMTTDTSTSTAYMELRSLRSDDTAVYYCARDLFPTIFGVSYYYYWGQGTLVTVSSASTKGPSVFPLAPSSKSTSGGTAALGCLVKDYFPEPVTVSWNSGALTSGVHTFPAVLQSSGLYSLSSVVTVPSSSLGTQTYICNVNHKPSNTKVDKKVEPKSCDKTHTCPPCPAPEAAGGPSVFLFPPKPKDTLMISRTPEVTCVVVDVSHEDPEVKFNWYVDGVEVHNAKTKPREEQYNSTYRVVSVLTVLHQDWLNGKEYKCKVSNKALPAPIEKTISKAKGQPREPQVYTLPPSRDELPYIIPPYNQVSLTCLVKGFYPSDIAVEWESNGQPENNYKTTPPVLDSDGSFFLYSKLTVGADRWLEGNVFSCSVMHEALHNHYTQKSLSLSPG

SEQ ID NO: 86 - protein, 214 aa, Artificial Sequence; identical to SEQ ID NO: 48
  FS22-172-003AA/G12v2 mAb2 light chain

SEQ ID NO: 87 - protein, 457 aa, Artificial Sequence
  FS22-172-003AA/G12v2 mAb2 heavy chain with LALA
EVQLVQSGAEVKRPGASVKVSCKASGYTFTSYGISWVRQAPGQGLEWMGWISAYSGGTNYAQKLQGRVTMTTDTSTSTAYMELRSLRSDDTAVYYCARDLFPTIFGVSYYYYWGQGTLVTVSSASTKGPSVFPLAPSSKSTSGGTAALGCLVKDYFPEPVTVSWNSGALTSGVHTFPAVLQSSGLYSLSSVVTVPSSSLGTQTYICNVNHKPSNTKVDKKVEPKSCDKTHTCPPCPAPEAAGGPSVFLFPPKPKDTLMISRTPEVTCVVVDVSHEDPEVKFNWYVDGVEVHNAKTKPREEQYNSTYRVVSVLTVLHQDWLNGKEYKCKVSNKALPAPIEKTISKAKGQPREPQVYTLPPSRDELPYIIPPYNQVSLTCLVKGFYPSDIAVEWESNGQPENNYKTTPPVLDSDGSFFLYSKLTVGADRWLEGNVFSCSVMHEALHNHYTQKSLSLSPG

SEQ ID NO: 88 - protein, 214 aa, Artificial Sequence; identical to SEQ ID NO: 50
  FS22-172-003AA/G12v2 mAb2 light chain

SEQ ID NO: 89 - protein, 457 aa, Artificial Sequence; identical to SEQ ID NO: 87
  FS22-172-003AA/E05v2 mAb2 heavy chain with LALA

SEQ ID NO: 90 - protein, 215 aa, Artificial Sequence; identical to SEQ ID NO: 52
  FS22-172-003AA/E05v2 mAb2 light chain

SEQ ID NO: 91 - protein, 457 aa, Artificial Sequence; identical to SEQ ID NO: 87
  FS22-172-003AA/lambdav3 mAb2 heavy chain with LALA

SEQ ID NO: 92 - protein, 217 aa, Artificial Sequence; identical to SEQ ID NO: 62
  FS22-172-003AA/lambdav3 mAb2 light chain

SEQ ID NO: 93 - protein, 452 aa, Artificial Sequence
  G1/280_02_G02 heavy chain with LALA
EVQLVQSGAEVKRPGASVKVSCKASGYTFTSYGISWVRQAPGQGLEWMGWISAYNGNTNYAQKLQGRVTMTTDTSTSTAYMELRSLRSDDTAVYYCARDLFPTIFGVSYYYYWGQGTLVTVSSASTKGPSVFPLAPSSKSTSGGTAALGCLVKDYFPEPVTVSWNSGALTSGVHTFPAVLQSSGLYSLSSVVTVPSSSLGTQTYICNVNHKPSNTKVDKKVEPKSCDKTHTCPPCPAPEAAGGPSVFLFPPKPKDTLMISRTPEVTCVVVDVSHEDPEVKFNWYVDGVEVHNAKTKPREEQYNSTYRVVSVLTVLHQDWLNGKEYKCKVSNKALPAPIEKTISKAKGQPREPQVYTLPPSRDELTKNQVSLTCLVKGFYPSDIAVEWESNGQPENNYKTTPPVLDSDGSFFLYSKLTVDKSRWQQGNVFSCSVMHEALHNHYTQKSLSLSPG

SEQ ID NO: 94 - protein, 8 aa, Artificial Sequence
  HCDR1 (IMGT)
GYTFTSYG

SEQ ID NO: 95 - protein, 8 aa, Artificial Sequence
  HCDR2 (IMGT) for G1/280_02_G02
ISAYNGNT

SEQ ID NO: 96 - protein, 9 aa, Artificial Sequence
  LCDR1 (IMGT) for G1/280_02_G02 and G1/280_02_G02_NS
SSDVGGYNS

SEQ ID NO: 97 - protein, 452 aa, Artificial Sequence
  G1/280_02_G02_NS heavy chain with LALA
EVQLVQSGAEVKRPGASVKVSCKASGYTFTSYGISWVRQAPGQGLEWMGWISAYNSNTNYAQKLQGRVTMTTDTSTSTAYMELRSLRSDDTAVYYCARDLFPTIFGVSYYYYWGQGTLVTVSSASTKGPSVFPLAPSSKSTSGGTAALGCLVKDYFPEPVTVSWNSGALTSGVHTFPAVLQSSGLYSLSSVVTVPSSSLGTQTYICNVNHKPSNTKVDKKVEPKSCDKTHTCPPCPAPEAAGGPSVFLFPPKPKDTLMISRTPEVTCVVVDVSHEDPEVKFNWYVDGVEVHNAKTKPREEQYNSTYRVVSVLTVLHQDWLNGKEYKCKVSNKALPAPIEKTISKAKGQPREPQVYTLPPSRDELTKNQVSLTCLVKGFYPSDIAVEWESNGQPENNYKTTPPVLDSDGSFFLYSKLTVDKSRWQQGNVFSCSVMHEALHNHYTQKSLSLSPG

SEQ ID NO: 98 - protein, 8 aa, Artificial Sequence
  HCDR2 (IMGT) for G1/280_02_G02_NS, G1/894_08_E05, G1/887_04_E12, G1/887_04_G12 and G1/894_08_A05
ISAYNSNT

SEQ ID NO: 99 - protein, 452 aa, Artificial Sequence; identical to SEQ ID NO: 97
  G1/894_08_E05 heavy chain with LALA

SEQ ID NO: 100 - protein, 6 aa, Artificial Sequence
  LCDR1 (IMGT)
QSISGR

SEQ ID NO: 101 - protein, 452 aa, Artificial Sequence
  G1/887_04_E12 heavy chain with LALA
EVQLVQSGAEVKRPGASVKVSCKASGYPFTSYGISWVRQAPGQGLEWMGWISAYNSNTNYAQKLQGRVTMTTDTSTSTAYMELRSLRSDDTAVYYCARDLFPTIFGVSYYYYWGQGTLVTVSSASTKGPSVFPLAPSSKSTSGGTAALGCLVKDYFPEPVTVSWNSGALTSGVHTFPAVLQSSGLYSLSSVVTVPSSSLGTQTYICNVNHKPSNTKVDKKVEPKSCDKTHTCPPCPAPEAAGGPSVFLFPPKPKDTLMISRTPEVTCVVVDVSHEDPEVKFNWYVDGVEVHNAKTKPREEQYNSTYRVVSVLTVLHQDWLNGKEYKCKVSNKALPAPIEKTISKAKGQPREPQVYTLPPSRDELTKNQVSLTCLVKGFYPSDIAVEWESNGQPENNYKTTPPVLDSDGSFFLYSKLTVDKSRWQQGNVFSCSVMHEALHNHYTQKSLSLSPG

SEQ ID NO: 102 - protein, 8 aa, Artificial Sequence
  HCDR1 (IMGT) of G1/887_04_E12, G1AA/E12v2, G1/929_01_A01, G1/929_01_A02 and G1/929_01_A03.
GYPFTSYG

SEQ ID NO: 103 - protein, 6 aa, Artificial Sequence
  LCDR1 (IMGT) G1/887_04_E12, G1AA/E12v2, G1/929_01_A01, G1/929_01_A02 and G1/929_01_A03.
QSIGNR

SEQ ID NO: 104 - protein, 452 aa, Artificial Sequence; identical to SEQ ID NO: 97
  G1/887_04_G12 heavy chain with LALA

SEQ ID NO: 105 - protein, 452 aa, Artificial Sequence; identical to SEQ ID NO: 97
  G1/894_08_A05 heavy chain with LALA

SEQ ID NO: 106 - protein, 4 aa, Artificial Sequence
  LCDR2 (IMGT) of G1/894_08_A05, G1/929_01_A10, G1/929_01_A11, G1/929_01_A12, G1/929_01_A04, G1/929_01_A05, and G1/929_01_A06.
EASN

SEQ ID NO: 107 - protein, 452 aa, Artificial Sequence
  G1AA/E05v2  heavy chain
EVQLVQSGAEVKRPGASVKVSCKASGYTFTSYGISWVRQAPGQGLEWMGWISAYSGGTNYAQKLQGRVTMTTDTSTSTAYMELRSLRSDDTAVYYCARDLFPTIFGVSYYYYWGQGTLVTVSSASTKGPSVFPLAPSSKSTSGGTAALGCLVKDYFPEPVTVSWNSGALTSGVHTFPAVLQSSGLYSLSSVVTVPSSSLGTQTYICNVNHKPSNTKVDKKVEPKSCDKTHTCPPCPAPELLGGPSVFLFPPKPKDTLMISRTPEVTCVVVDVSHEDPEVKFNWYVDGVEVHNAKTKPREEQYNSTYRVVSVLTVLHQDWLNGKEYKCKVSNKALPAPIEKTISKAKGQPREPQVYTLPPSRDELTKNQVSLTCLVKGFYPSDIAVEWESNGQPENNYKTTPPVLDSDGSFFLYSKLTVDKSRWQQGNVFSCSVMHEALHNHYTQKSLSLSPG

SEQ ID NO: 108 - DNA, 1356 bp, Artificial Sequence
  G1AA/E05v2 heavy chain DNA
gaagtgcagctggtgcagtccggagccgaagtcaagaggcctggagcgtccgtgaaggtgtcctgcaaagcctcaggatacaccttcacttcgtacgggatttcctgggtccgccaagcaccgggtcaaggcttggagtggatgggatggatcagcgcgtattccgggggaaccaactacgctcaaaagctgcagggtcgcgtgaccatgaccaccgatacctccacctcaacggcctacatggaactgagatctctgcggagcgacgacactgccgtgtactactgtgcccgggacctgttccccactatcttcggagtgtcgtactactactactggggccaggggactctcgtgaccgtgtcgagcgctagcactaagggcccgtcggtgttcccgctggccccatcgtccaagagcacatcagggggtaccgccgccctgggctgccttgtgaaggattactttcccgagcccgtcacagtgtcctggaacagcggagccctgacctccggagtgcatactttcccggctgtgcttcagtcctctggcctgtactcattgtcctccgtggtcaccgtcccttcgtcctccctgggcacccagacctatatctgtaatgtcaaccataagccctcgaacaccaaggtcgacaagaaggtcgagccgaagtcgtgcgacaagactcacacttgcccgccttgcccagccccggaactgctgggtggtccttcggtgttcctcttcccgcccaagccgaaggataccctgatgatctcacggacccccgaagtgacctgtgtggtggtggacgtgtcccacgaggacccggaagtgaaattcaattggtacgtggatggagtggaagtgcacaacgccaagaccaagccacgggaagaacagtacaactctacctaccgcgtggtgtccgtgctcactgtgctgcaccaagactggctgaacgggaaggagtacaagtgcaaagtgtccaacaaggcgctgcctgccccaattgagaaaactatctcgaaagccaagggacagcctcgagagcctcaagtgtacaccctgcctccctctcgggacgagctgaccaagaaccaagtctccctgacctgtctggtcaagggattctacccatcggatatcgccgtggaatgggaaagcaacggacagcccgagaacaactacaagacgactccgcccgtgctggattccgacgggagcttcttcttgtactccaagctgaccgtcgacaagagcagatggcagcagggaaacgtgttctcctgctccgtgatgcatgaggcgctgcacaaccactacactcagaagagcttgtccctgtcgcccgga

SEQ ID NO: 109 - DNA, 1356 bp, Artificial Sequence
  G1AA/E05v2 heavy chain DNA (with LALA)
gaagtgcagctggtgcagtccggagccgaagtcaagaggcctggagcgtccgtgaaggtgtcctgcaaagcctcaggatacaccttcacttcgtacgggatttcctgggtccgccaagcaccgggtcaaggcttggagtggatgggatggatcagcgcgtattccgggggaaccaactacgctcaaaagctgcagggtcgcgtgaccatgaccaccgatacctccacctcaacggcctacatggaactgagatctctgcggagcgacgacactgccgtgtactactgtgcccgggacctgttccccactatcttcggagtgtcgtactactactactggggccaggggactctcgtgaccgtgtcgagcgctagcactaagggcccgtcggtgttcccgctggccccatcgtccaagagcacatcagggggtaccgccgccctgggctgccttgtgaaggattactttcccgagcccgtcacagtgtcctggaacagcggagccctgacctccggagtgcatactttcccggctgtgcttcagtcctctggcctgtactcattgtcctccgtggtcaccgtcccttcgtcctccctgggcacccagacctatatctgtaatgtcaaccataagccctcgaacaccaaggtcgacaagaaggtcgagccgaagtcgtgcgacaagactcacacttgcccgccttgcccagccccggaagctgccggtggtccttcggtgttcctcttcccgcccaagccgaaggataccctgatgatctcacggacccccgaagtgacctgtgtggtggtggacgtgtcccacgaggacccggaagtgaaattcaattggtacgtggatggagtggaagtgcacaacgccaagaccaagccacgggaagaacagtacaactctacctaccgcgtggtgtccgtgctcactgtgctgcaccaagactggctgaacgggaaggagtacaagtgcaaagtgtccaacaaggcgctgcctgccccaattgagaaaactatctcgaaagccaagggacagcctcgagagcctcaagtgtacaccctgcctccctctcgggacgagctgaccaagaaccaagtctccctgacctgtctggtcaagggattctacccatcggatatcgccgtggaatgggaaagcaacggacagcccgagaacaactacaagacgactccgcccgtgctggattccgacgggagcttcttcttgtactccaagctgaccgtcgacaagagcagatggcagcagggaaacgtgttctcctgctccgtgatgcatgaggcgctgcacaaccactacactcagaagagcttgtccctgtcgcccgga

SEQ ID NO: 110 - DNA, 369 bp, Artificial Sequence
  G1AA/E05v2 VH domain DNA
gaagtgcagctggtgcagtccggagccgaagtcaagaggcctggagcgtccgtgaaggtgtcctgcaaagcctcaggatacaccttcacttcgtacgggatttcctgggtccgccaagcaccgggtcaaggcttggagtggatgggatggatcagcgcgtattccgggggaaccaactacgctcaaaagctgcagggtcgcgtgaccatgaccaccgatacctccacctcaacggcctacatggaactgagatctctgcggagcgacgacactgccgtgtactactgtgcccgggacctgttccccactatcttcggagtgtcgtactactactactggggccaggggactctcgtgaccgtgtcgagc

SEQ ID NO: 111 - protein, 8 aa, Artificial Sequence
  HCDR2 (IMGT) G1AA/E05v2, G1AA/E12v2, G1AA/G12v2, G1AA/lambdav3, G1/929_01_A08, G1/929_01_A02, G1/929_01_A11 and G1/929_01_A05.
ISAYSGGT

SEQ ID NO: 112 - DNA, 645 bp, Artificial Sequence
  G1AA/E05v2 Light chain DNA
gacattcagatgacccaatccccgtccacgctgagcgcctccgtcggtgatcgcgtgacaatcacttgtcgggcgtcgcagtccatctctggaaggctcgcctggtaccagcagaagcctggaaaggctcccaacctccttatctacgaagccagcaacctggagtccggagtgcctagccggttcagcggatcagggtccggtaccgagttcaccctgaccatttcctcgctccaacctgaggacttcgccacctactactgccaacagtcctattcaactccgcgcgtgaccttcggccagggcactaaggtcgaaatcaaaagaaccgtggcagccccatcggtgtttatcttcccgccctcggacgaacagctgaagtcaggcactgctagcgtggtctgtctcctgaacaatttctacccgcgcgaagctaaggtccagtggaaggtcgacaacgcgctgcagtccggaaacagccaggagtcagtgaccgagcaggactccaaggattccacttattccctgtcctccaccctgactttgagcaaggccgactacgagaagcacaaagtgtacgcctgcgaagtgacccatcaagggctttcgtcgcccgtgaccaagagcttcaaccggggcgaatgc

SEQ ID NO: 113 - DNA, 324 bp, Artificial Sequence
  G1AA/E05v2 VL domain DNA
gacattcagatgacccaatccccgtccacgctgagcgcctccgtcggtgatcgcgtgacaatcacttgtcgggcgtcgcagtccatctctggaaggctcgcctggtaccagcagaagcctggaaaggctcccaacctccttatctacgaagccagcaacctggagtccggagtgcctagccggttcagcggatcagggtccggtaccgagttcaccctgaccatttcctcgctccaacctgaggacttcgccacctactactgccaacagtcctattcaactccgcgcgtgaccttcggccagggcactaaggtcgaaatcaaa

SEQ ID NO: 114 - protein, 452 aa, Artificial Sequence
  G1AA/E12v2 Heavy chain
EVQLVQSGAEVKRPGASVKVSCKASGYPFTSYGISWVRQAPGQGLEWMGWISAYSGGTNYAQKLQGRVTMTTDTSTSTAYMELRSLRSDDTAVYYCARDLFPTIFGVSYYYYWGQGTLVTVSSASTKGPSVFPLAPSSKSTSGGTAALGCLVKDYFPEPVTVSWNSGALTSGVHTFPAVLQSSGLYSLSSVVTVPSSSLGTQTYICNVNHKPSNTKVDKKVEPKSCDKTHTCPPCPAPELLGGPSVFLFPPKPKDTLMISRTPEVTCVVVDVSHEDPEVKFNWYVDGVEVHNAKTKPREEQYNSTYRVVSVLTVLHQDWLNGKEYKCKVSNKALPAPIEKTISKAKGQPREPQVYTLPPSRDELTKNQVSLTCLVKGFYPSDIAVEWESNGQPENNYKTTPPVLDSDGSFFLYSKLTVDKSRWQQGNVFSCSVMHEALHNHYTQKSLSLSPG

SEQ ID NO: 115 - DNA, 1356 bp, Artificial Sequence
  G1AA/E12v2 heavy chain DNA
gaagtgcagctggtgcagtccggagccgaagtcaagaggcctggagcgtccgtgaaggtgtcctgcaaagcctcaggataccccttcacttcgtacgggatttcctgggtccgccaagcaccgggtcaaggcttggagtggatgggatggatcagcgcgtattccgggggaaccaactacgctcaaaagctgcagggtcgcgtgaccatgaccaccgatacctccacctcaacggcctacatggaactgagatctctgcggagcgacgacactgccgtgtactactgtgcccgggacctgttccccactatcttcggagtgtcgtactactactactggggccaggggactctcgtgaccgtgtcgagcgctagcactaagggcccgtcggtgttcccgctggccccatcgtccaagagcacatcagggggtaccgccgccctgggctgccttgtgaaggattactttcccgagcccgtcacagtgtcctggaacagcggagccctgacctccggagtgcatactttcccggctgtgcttcagtcctctggcctgtactcattgtcctccgtggtcaccgtcccttcgtcctccctgggcacccagacctatatctgtaatgtcaaccataagccctcgaacaccaaggtcgacaagaaggtcgagccgaagtcgtgcgacaagactcacacttgcccgccttgcccagccccggaactgctgggtggtccttcggtgttcctcttcccgcccaagccgaaggataccctgatgatctcacggacccccgaagtgacctgtgtggtggtggacgtgtcccacgaggacccggaagtgaaattcaattggtacgtggatggagtggaagtgcacaacgccaagaccaagccacgggaagaacagtacaactctacctaccgcgtggtgtccgtgctcactgtgctgcaccaagactggctgaacgggaaggagtacaagtgcaaagtgtccaacaaggcgctgcctgccccaattgagaaaactatctcgaaagccaagggacagcctcgagagcctcaagtgtacaccctgcctccctctcgggacgagctgaccaagaaccaagtctccctgacctgtctggtcaagggattctacccatcggatatcgccgtggaatgggaaagcaacggacagcccgagaacaactacaagacgactccgcccgtgctggattccgacgggagcttcttcttgtactccaagctgaccgtcgacaagagcagatggcagcagggaaacgtgttctcctgctccgtgatgcatgaggcgctgcacaaccactacactcagaagagcttgtccctgtcgcccgga

SEQ ID NO: 116 - DNA, 1356 bp, Artificial Sequence
  G1AA/E12v2 (with LALA) heavy chain DNA
gaagtgcagctggtgcagtccggagccgaagtcaagaggcctggagcgtccgtgaaggtgtcctgcaaagcctcaggataccccttcacttcgtacgggatttcctgggtccgccaagcaccgggtcaaggcttggagtggatgggatggatcagcgcgtattccgggggaaccaactacgctcaaaagctgcagggtcgcgtgaccatgaccaccgatacctccacctcaacggcctacatggaactgagatctctgcggagcgacgacactgccgtgtactactgtgcccgggacctgttccccactatcttcggagtgtcgtactactactactggggccaggggactctcgtgaccgtgtcgagcgctagcactaagggcccgtcggtgttcccgctggccccatcgtccaagagcacatcagggggtaccgccgccctgggctgccttgtgaaggattactttcccgagcccgtcacagtgtcctggaacagcggagccctgacctccggagtgcatactttcccggctgtgcttcagtcctctggcctgtactcattgtcctccgtggtcaccgtcccttcgtcctccctgggcacccagacctatatctgtaatgtcaaccataagccctcgaacaccaaggtcgacaagaaggtcgagccgaagtcgtgcgacaagactcacacttgcccgccttgcccagccccggaagctgccggtggtccttcggtgttcctcttcccgcccaagccgaaggataccctgatgatctcacggacccccgaagtgacctgtgtggtggtggacgtgtcccacgaggacccggaagtgaaattcaattggtacgtggatggagtggaagtgcacaacgccaagaccaagccacgggaagaacagtacaactctacctaccgcgtggtgtccgtgctcactgtgctgcaccaagactggctgaacgggaaggagtacaagtgcaaagtgtccaacaaggcgctgcctgccccaattgagaaaactatctcgaaagccaagggacagcctcgagagcctcaagtgtacaccctgcctccctctcgggacgagctgaccaagaaccaagtctccctgacctgtctggtcaagggattctacccatcggatatcgccgtggaatgggaaagcaacggacagcccgagaacaactacaagacgactccgcccgtgctggattccgacgggagcttcttcttgtactccaagctgaccgtcgacaagagcagatggcagcagggaaacgtgttctcctgctccgtgatgcatgaggcgctgcacaaccactacactcagaagagcttgtccctgtcgcccgga

SEQ ID NO: 117 - DNA, 369 bp, Artificial Sequence
  G1AA/E12v2 VH domain DNA
gaagtgcagctggtgcagtccggagccgaagtcaagaggcctggagcgtccgtgaaggtgtcctgcaaagcctcaggataccccttcacttcgtacgggatttcctgggtccgccaagcaccgggtcaaggcttggagtggatgggatggatcagcgcgtattccgggggaaccaactacgctcaaaagctgcagggtcgcgtgaccatgaccaccgatacctccacctcaacggcctacatggaactgagatctctgcggagcgacgacactgccgtgtactactgtgcccgggacctgttccccactatcttcggagtgtcgtactactactactggggccaggggactctcgtgaccgtgtcgagc

SEQ ID NO: 118 - DNA, 642 bp, Artificial Sequence
  G1AA/E12v2 light chain DNA
gacatccagatgacgcagagcccgtctaccctgtccgcctccgtgagagatcgcgtgatcatcacctgtcgggccagccagtccatcggaaaccgcttggcgtggtaccagcacaagcctgggaaggctccgaagctgctcatctacgaagcctcgacttcggagactggtgtccctagccggttcagcggatcgggatcagggaccgatttcactctgaccatttcctccctgcaacccgaggacttcgccacctactactgccaacagtcatattccaccccgtacaccttcggacaaggcaccaagctcgaaatcaagcggactgtcgccgcaccttccgtgttcattttcccaccctccgacgaacagctgaaatcgggtacagctagcgtggtctgtctcctgaacaatttctacccgcgcgaagctaaggtccagtggaaggtcgacaacgcgctgcagtccggaaacagccaggagtcagtgaccgagcaggactccaaggattccacttattccctgtcctccaccctgactttgagcaaggccgactacgagaagcacaaagtgtacgcctgcgaagtgacccatcaagggctttcgtcgcccgtgaccaagagcttcaaccggggcgaatgc

SEQ ID NO: 119 - DNA, 321 bp, Artificial Sequence
  G1AA/E12v2 VL domain DNA
gacatccagatgacgcagagcccgtctaccctgtccgcctccgtgagagatcgcgtgatcatcacctgtcgggccagccagtccatcggaaaccgcttggcgtggtaccagcacaagcctgggaaggctccgaagctgctcatctacgaagcctcgacttcggagactggtgtccctagccggttcagcggatcgggatcagggaccgatttcactctgaccatttcctccctgcaacccgaggacttcgccacctactactgccaacagtcatattccaccccgtacaccttcggacaaggcaccaagctcgaaatcaag

SEQ ID NO: 120 - protein, 452 aa, Artificial Sequence; identical to SEQ ID NO: 107
  G1AA/G12v2 heavy chain

SEQ ID NO: 121 - DNA, 1356 bp, Artificial Sequence; identical to SEQ ID NO: 108
  G1AA/G12v2 heavy chain DNA

SEQ ID NO: 122 - DNA, 1356 bp, Artificial Sequence; identical to SEQ ID NO: 109
  G1AA/G12v2 LALA heavy chain DNA

SEQ ID NO: 123 - DNA, 369 bp, Artificial Sequence; identical to SEQ ID NO: 110
  G1AA/G12v2 VH domain DNA

SEQ ID NO: 124 - DNA, 642 bp, Artificial Sequence
  G1AA/G12v2 light chain DNA
gacattcagatgacccagtccccgagcacgctgtccgcaagcgtgggggacagagtgaccatcacttgccgcgcctcacaatccatcagcggacgcttggcctggtaccagcagaagcccggaaaggccccaaaccttctgatctacgaagcctcgaacctggagtcaggcgtcccttcgcggttctctggctccggttccggaactgagttcaccctcaccatctcgtccctgcaaccggaagatttcgccacctactactgccaacagtcgtactcctggccccggacattcggacagggaaccaaagtcgagattaagcggactgtggcggctcctagcgtgttcatctttcccccgtccgacgaacagctgaagtccggtaccgctagcgtggtctgtctcctgaacaatttctacccgcgcgaagctaaggtccagtggaaggtcgacaacgcgctgcagtccggaaacagccaggagtcagtgaccgagcaggactccaaggattccacttattccctgtcctccaccctgactttgagcaaggccgactacgagaagcacaaagtgtacgcctgcgaagtgacccatcaagggctttcgtcgcccgtgaccaagagcttcaaccggggcgaatgc

SEQ ID NO: 125 - DNA, 321 bp, Artificial Sequence
  G1AA/G12v2 VL domain DNA
gacattcagatgacccagtccccgagcacgctgtccgcaagcgtgggggacagagtgaccatcacttgccgcgcctcacaatccatcagcggacgcttggcctggtaccagcagaagcccggaaaggccccaaaccttctgatctacgaagcctcgaacctggagtcaggcgtcccttcgcggttctctggctccggttccggaactgagttcaccctcaccatctcgtccctgcaaccggaagatttcgccacctactactgccaacagtcgtactcctggccccggacattcggacagggaaccaaagtcgagattaag

SEQ ID NO: 126 - protein, 452 aa, Artificial Sequence; identical to SEQ ID NO: 107
  G1AA/lambdav3 heavy chain

SEQ ID NO: 127 - DNA, 1356 bp, Artificial Sequence; identical to SEQ ID NO: 108
  G1AA/lambdav3 heavy chain DNA

SEQ ID NO: 128 - DNA, 1356 bp, Artificial Sequence; identical to SEQ ID NO: 109
  G1AA/lambdav3 with LALA heavy chain DNA

SEQ ID NO: 129 - DNA, 369 bp, Artificial Sequence; identical to SEQ ID NO: 110
  G1AA/lambdav3 VH domain DNA

SEQ ID NO: 130 - DNA, 651 bp, Artificial Sequence
  G1AA/lambdav3 light chain DNA
cagtcggcccttactcaacccgcgtcagtctccggtagccccggacagtccatcacgatttcgtgcaccggaaccagcagcgatgtcgggggatacaactacgtgtcctggtaccagcagttcccgggaaaggcccctaagctgatgatcttcgaagtcactaacagaccttccggagtgtcggaccggttctccggctccaagtccgacaacactgcgagcctgaccatctcgggcctgcaagccgaggacgaagccgagtactactgtagctcattcaagcgcggttccaccctcgtggtgttcggcggtggcactaagctcaccgtgctgggacagccagccgcagctcctagcgtgaccttgttccccccgtcgagcgaagaactgcaggccaacaaggccaccctcgtctgcctgatctccgacttctaccctggggccgtgactgtggcttggaaggccgattcaagcccagtgaaagccggagtggaaaccaccactccgtccaagcagtcgaacaataagtatgccgcgtcctcctacctgtcgctgaccccggagcagtggaagtcccatcggtcctactcctgccaagtcacccacgaagggtccactgtggagaaaacagtggctcccaccgagtgctct

SEQ ID NO: 131 - DNA, 336 bp, Artificial Sequence
  G1AA/lambdav3 VL DNA
cagtcggcccttactcaacccgcgtcagtctccggtagccccggacagtccatcacgatttcgtgcaccggaaccagcagcgatgtcgggggatacaactacgtgtcctggtaccagcagttcccgggaaaggcccctaagctgatgatcttcgaagtcactaacagaccttccggagtgtcggaccggttctccggctccaagtccgacaacactgcgagcctgaccatctcgggcctgcaagccgaggacgaagccgagtactactgtagctcattcaagcgcggttccaccctcgtggtgttcggcggtggcactaagctcaccgtgctggga

SEQ ID NO: 132 - protein, 9 aa, Artificial Sequence
  G1AA/lambdav3 LCDR1 (IMGT)
SSDVGGYNY

SEQ ID NO: 133 - protein, 452 aa, Artificial Sequence
  G1/929_01_A07 heavy chain
EVQLVQSGAEVKRPGASVKVSCKASGYTFTSYGISWVRQAPGQGLEWMGWISAYGGSTNYAQKLQGRVTMTTDTSTSTAYMELRSLRSDDTAVYYCARDLFPTIFGVSYYYYWGQGTLVTVSSASTKGPSVFPLAPSSKSTSGGTAALGCLVKDYFPEPVTVSWNSGALTSGVHTFPAVLQSSGLYSLSSVVTVPSSSLGTQTYICNVNHKPSNTKVDKKVEPKSCDKTHTCPPCPAPELLGGPSVFLFPPKPKDTLMISRTPEVTCVVVDVSHEDPEVKFNWYVDGVEVHNAKTKPREEQYNSTYRVVSVLTVLHQDWLNGKEYKCKVSNKALPAPIEKTISKAKGQPREPQVYTLPPSRDELTKNQVSLTCLVKGFYPSDIAVEWESNGQPENNYKTTPPVLDSDGSFFLYSKLTVDKSRWQQGNVFSCSVMHEALHNHYTQKSLSLSPG

SEQ ID NO: 134 - protein, 123 aa, Artificial Sequence
  G1/929_01_A07 VH domain
EVQLVQSGAEVKRPGASVKVSCKASGYTFTSYGISWVRQAPGQGLEWMGWISAYGGSTNYAQKLQGRVTMTTDTSTSTAYMELRSLRSDDTAVYYCARDLFPTIFGVSYYYYWGQGTLVTVSS

SEQ ID NO: 135 - protein, 8 aa, Artificial Sequence
  HCDR2 (IMGT) of G1/929_01_A07 , G1/929_01_A01, G1/929_01_A10 and G1/929_01_A04
ISAYGGST

SEQ ID NO: 136 - protein, 17 aa, Artificial Sequence
  HCDR2 (Kabat) of G1/929_01_A07, G1/929_01_A01, G1/929_01_A10 and G1/929_01_A04.
WISAYGGSTNYAQKLQG

SEQ ID NO: 137 - protein, 216 aa, Artificial Sequence; identical to SEQ ID NO: 58
  G1/929_01_A07 light chain

SEQ ID NO: 138 - protein, 108 aa, Artificial Sequence; identical to SEQ ID NO: 32
  G1/929_01_A07 VL domain

SEQ ID NO: 139 - protein, 452 aa, Artificial Sequence; identical to SEQ ID NO: 107
  G1/929_01_A08 heavy chain

SEQ ID NO: 140 - protein, 123 aa, Artificial Sequence; identical to SEQ ID NO: 29
  G1/929_01_A08 VH domain

SEQ ID NO: 141 - protein, 216 aa, Artificial Sequence; identical to SEQ ID NO: 58
  G1/929_01_A08 light chain

SEQ ID NO: 142 - protein, 108 aa, Artificial Sequence; identical to SEQ ID NO: 32
  G1/929_01_A08 VL domain

SEQ ID NO: 143 - protein, 452 aa, Artificial Sequence
  G1/929_01_A09 heavy chain
EVQLVQSGAEVKRPGASVKVSCKASGYTFTSYGISWVRQAPGQGLEWMGWISAYSGNANYAQKLQGRVTMTTDTSTSTAYMELRSLRSDDTAVYYCARDLFPTIFGVSYYYYWGQGTLVTVSSASTKGPSVFPLAPSSKSTSGGTAALGCLVKDYFPEPVTVSWNSGALTSGVHTFPAVLQSSGLYSLSSVVTVPSSSLGTQTYICNVNHKPSNTKVDKKVEPKSCDKTHTCPPCPAPELLGGPSVFLFPPKPKDTLMISRTPEVTCVVVDVSHEDPEVKFNWYVDGVEVHNAKTKPREEQYNSTYRVVSVLTVLHQDWLNGKEYKCKVSNKALPAPIEKTISKAKGQPREPQVYTLPPSRDELTKNQVSLTCLVKGFYPSDIAVEWESNGQPENNYKTTPPVLDSDGSFFLYSKLTVDKSRWQQGNVFSCSVMHEALHNHYTQKSLSLSPG

SEQ ID NO: 144 - protein, 123 aa, Artificial Sequence
  G1/929_01_A09 VH domain
EVQLVQSGAEVKRPGASVKVSCKASGYTFTSYGISWVRQAPGQGLEWMGWISAYSGNANYAQKLQGRVTMTTDTSTSTAYMELRSLRSDDTAVYYCARDLFPTIFGVSYYYYWGQGTLVTVSS

SEQ ID NO: 145 - protein, 8 aa, Artificial Sequence
  HCDR2 (IMGT) of G1/929_01_A09, G1/929_01_A03, G1/929_01_A12 and G1/929_01_A06.
ISAYSGNA

SEQ ID NO: 146 - protein, 17 aa, Artificial Sequence
  HCDR2 (Kabat) of G1/929_01_A09, G1/929_01_A03, G1/929_01_A12 and G1/929_01_A12
WISAYSGNANYAQKLQG

SEQ ID NO: 147 - protein, 216 aa, Artificial Sequence; identical to SEQ ID NO: 58
  G1/929_01_A09 light chain

SEQ ID NO: 148 - protein, 108 aa, Artificial Sequence; identical to SEQ ID NO: 32
  G1/929_01_A09 VL domain

SEQ ID NO: 149 - protein, 452 aa, Artificial Sequence; identical to SEQ ID NO: 133
  G1/929_01_A01 heavy chain

SEQ ID NO: 150 - protein, 123 aa, Artificial Sequence
  G1/929_01_A01 VH domain
EVQLVQSGAEVKRPGASVKVSCKASGYPFTSYGISWVRQAPGQGLEWMGWISAYGGSTNYAQKLQGRVTMTTDTSTSTAYMELRSLRSDDTAVYYCARDLFPTIFGVSYYYYWGQGTLVTVSS

SEQ ID NO: 151 - protein, 215 aa, Artificial Sequence; identical to SEQ ID NO: 54
  G1/929_01_A01 light chain

SEQ ID NO: 152 - protein, 107 aa, Artificial Sequence; identical to SEQ ID NO: 28
  G1/929_01_A01 VL domain

SEQ ID NO: 153 - protein, 452 aa, Artificial Sequence; identical to SEQ ID NO: 107
  G1/929_01_A02 heavy chain

SEQ ID NO: 154 - protein, 123 aa, Artificial Sequence; identical to SEQ ID NO: 27
  G1/929_01_A02 VH domain

SEQ ID NO: 155 - protein, 215 aa, Artificial Sequence; identical to SEQ ID NO: 54
  G1/929_01_A02 light chain

SEQ ID NO: 156 - protein, 107 aa, Artificial Sequence; identical to SEQ ID NO: 28
  G1/929_01_A02 VL domain

SEQ ID NO: 157 - protein, 452 aa, Artificial Sequence; identical to SEQ ID NO: 143
  G1/929_01_A03 heavy chain

SEQ ID NO: 158 - protein, 123 aa, Artificial Sequence
  G1/929_01_A03 VH domain
EVQLVQSGAEVKRPGASVKVSCKASGYPFTSYGISWVRQAPGQGLEWMGWISAYSGNANYAQKLQGRVTMTTDTSTSTAYMELRSLRSDDTAVYYCARDLFPTIFGVSYYYYWGQGTLVTVSS

SEQ ID NO: 159 - protein, 215 aa, Artificial Sequence; identical to SEQ ID NO: 54
  G1/929_01_A03 light chain

SEQ ID NO: 160 - protein, 107 aa, Artificial Sequence; identical to SEQ ID NO: 28
  G1/929_01_A03 VL domain

SEQ ID NO: 161 - protein, 452 aa, Artificial Sequence; identical to SEQ ID NO: 133
  G1/929_01_A10 heavy chain

SEQ ID NO: 162 - protein, 123 aa, Artificial Sequence; identical to SEQ ID NO: 134
  G1/929_01_A10 VH domain.

SEQ ID NO: 163 - protein, 215 aa, Artificial Sequence; identical to SEQ ID NO: 56
  G1/929_01_A10 light chain.

SEQ ID NO: 164 - protein, 107 aa, Artificial Sequence; identical to SEQ ID NO: 30
  G1/929_01_A10 VL domain.

SEQ ID NO: 165 - protein, 452 aa, Artificial Sequence; identical to SEQ ID NO: 107
  G1/929_01_A11 heavy chain

SEQ ID NO: 166 - protein, 215 aa, Artificial Sequence; identical to SEQ ID NO: 56
  G1/929_01_A11 light chain.

SEQ ID NO: 167 - protein, 107 aa, Artificial Sequence; identical to SEQ ID NO: 30
  G1/929_01_A11 VL domain.

SEQ ID NO: 168 - protein, 452 aa, Artificial Sequence; identical to SEQ ID NO: 143
  G1/929_01_A12 heavy chain.

SEQ ID NO: 169 - protein, 123 aa, Artificial Sequence; identical to SEQ ID NO: 144
  G1/929_01_A12 VH domain

SEQ ID NO: 170 - protein, 215 aa, Artificial Sequence; identical to SEQ ID NO: 56
  G1/929_01_A12 light chain

SEQ ID NO: 171 - protein, 107 aa, Artificial Sequence; identical to SEQ ID NO: 30
  G1/929_01_A12 VL domain.

SEQ ID NO: 172 - protein, 452 aa, Artificial Sequence; identical to SEQ ID NO: 133
  G1/929_01_A04 heavy chain.

SEQ ID NO: 173 - protein, 123 aa, Artificial Sequence; identical to SEQ ID NO: 134
  G1/929_01_A04 VH domain.

SEQ ID NO: 174 - protein, 216 aa, Artificial Sequence; identical to SEQ ID NO: 60
  G1/929_01_A04 light chain.

SEQ ID NO: 175 - protein, 108 aa, Artificial Sequence; identical to SEQ ID NO: 40
  G1/929_01_A04 VL domain.

SEQ ID NO: 176 - protein, 452 aa, Artificial Sequence; identical to SEQ ID NO: 107
  G1/929_01_A05 heavy chain.

SEQ ID NO: 177 - protein, 123 aa, Artificial Sequence; identical to SEQ ID NO: 29
  G1/929_01_A05 VH domain.

SEQ ID NO: 178 - protein, 216 aa, Artificial Sequence; identical to SEQ ID NO: 60
  G1/929_01_A05 light chain.

SEQ ID NO: 179 - protein, 108 aa, Artificial Sequence; identical to SEQ ID NO: 40
  G1/929_01_A05 VL domain.

SEQ ID NO: 180 - protein, 452 aa, Artificial Sequence; identical to SEQ ID NO: 143
  G1/929_01_A06 heavy chain.

SEQ ID NO: 181 - protein, 123 aa, Artificial Sequence; identical to SEQ ID NO: 144
  G1/929_01_A06 VH domain.

SEQ ID NO: 182 - protein, 216 aa, Artificial Sequence; identical to SEQ ID NO: 60
  G1/929_01_A06 light chain.

SEQ ID NO: 183 - protein, 108 aa, Artificial Sequence; identical to SEQ ID NO: 40
  G1/929_01_A06 VL domain.

SEQ ID NO: 184 - protein, 433 aa, Artificial Sequence
  Cynomolgus PD-L1-rCd4-His
MRIFAVFIFTIYWHLLNAFTVTVPKDLYVVEYGSNMTIECKFPVEKQLDLTSLIVYWEMEDKNIIQFVHGEEDLKVQHSNYRQRAQLLKDQLSLGNAALRITDVKLQDAGVYRCMISYGGADYKRITVKVNAPYNKINQRILVVDPVTSEHELTCQAEGYPKAEVIWTSSDHQVLSGKTTTTNSKREEKLLNVTSTLRINTTANEIFYCIFRRLDPEENHTAELVIPELPLALPPNERTAAATSITAYKSEGESAEFSFPLNLGEESLQGELRWKAEKAPSSQSWITFSLKNQKVSVQKSTSNPKFQLSETLPLTLQIPQVSLQFAGSGNLTLTLDRGILYQEVNLVVMKVTQPDSNTLTCEVMGPTSPKMRLILKQENQEARVSRQEKVIQVQAPEAGVWQCLLSEGEEVKMDSKIQVLSKGLNGSHHHHHH